European Patent Application EP 4 640 702 A1, published October 29, 2025. Title: Use of α-2,6-sialylated immunoglobulin for preventing or treating xerophthalmia or inflammatory ophthalmic diseases. Applicant: KONKUK UNIVERSITY INDUSTRIAL COOPERATION CORP. The sequence listing filed with the application follows.

SEQUENCE LISTING (14 sequences)

SEQ ID NO: 1 - DNA, 20 bp, synthetic construct
  source 1..20: mol_type = other DNA
tgtgcttcacgctgttcact

SEQ ID NO: 2 - DNA, 20 bp, synthetic construct
  source 1..20: mol_type = other DNA
ctcctcagcactttggacga

SEQ ID NO: 3 - DNA, 22 bp, synthetic construct
  source 1..22: mol_type = other DNA
tgacgacatcaagaaggtggtg

SEQ ID NO: 4 - DNA, 21 bp, synthetic construct
  source 1..21: mol_type = other DNA
gaaggtggaggagtgggtggc

SEQ ID NO: 5 - DNA, 20 bp, synthetic construct
  source 1..20: mol_type = other DNA
gagaaccacagtccagccat

SEQ ID NO: 6 - DNA, 20 bp, synthetic construct
  source 1..20: mol_type = other DNA
catggctttgtagacgcctt

SEQ ID NO: 7 - DNA, 19 bp, synthetic construct
  source 1..19: mol_type = other DNA
gagtacctgttccgctatg

SEQ ID NO: 8 - DNA, 23 bp, synthetic construct
  source 1..23: mol_type = other DNA
tgccacttgaggtcaccctcgaa

SEQ ID NO: 9 - DNA, 23 bp, synthetic construct
  source 1..23: mol_type = other DNA
tggctgaacaacacatagaactg

SEQ ID NO: 10 - DNA, 20 bp, synthetic construct
  source 1..20: mol_type = other DNA
acgcaggcagcaattatcct

SEQ ID NO: 11 - DNA, 20 bp, synthetic construct
  source 1..20: mol_type = other DNA
ctcccagacccaaaacacct

SEQ ID NO: 12 - DNA, 20 bp, synthetic construct
  source 1..20: mol_type = other DNA
ctggccttggggagcaaaag

SEQ ID NO: 13 - DNA, 20 bp, synthetic construct
  source 1..20: mol_type = other DNA
gtcaaggctgagaacgggaa

SEQ ID NO: 14 - DNA, 20 bp, synthetic construct
  source 1..20: mol_type = other DNA
ctccgatgcctgcttcacta